European Patent Application EP 4 660 205 A1, published December 10, 2025. Title: Mutiple antibodies against human IL-36R and/or human IL-1R3, and uses thereof. Applicant: Beijing Wisdomab Biotechnology Co., Ltd. Application EP. The sequence listing filed with the application follows.

SEQUENCE LISTING (56 sequences)

SEQ ID NO: 1 - protein, 5 aa, synthetic construct
SSWIH

SEQ ID NO: 2 - protein, 17 aa, synthetic construct
EINPGNVRSNYNENFRN

SEQ ID NO: 3 - protein, 10 aa, synthetic construct
INYGEPYFAS

SEQ ID NO: 4 - protein, 12 aa, synthetic construct
RASQSVIGSYLA

SEQ ID NO: 5 - protein, 7 aa, synthetic construct
SASKLAS

SEQ ID NO: 6 - protein, 9 aa, synthetic construct
QQDTRYPIT

SEQ ID NO: 7 - protein, 17 aa, synthetic construct
EINPGSGRSNYNENFQG

SEQ ID NO: 8 - protein, 10 aa, synthetic construct
VFYGEPYFPF

SEQ ID NO: 9 - protein, 12 aa, synthetic construct
RASQSVIYSYLA

SEQ ID NO: 10 - protein, 7 aa, synthetic construct
SASKRAS

SEQ ID NO: 11 - protein, 9 aa, synthetic construct
QQHAGIPVT

SEQ ID NO: 12 - protein, 5 aa, synthetic construct
SYAMS

SEQ ID NO: 13 - protein, 17 aa, synthetic construct
EISRGGSHTYYPDTVTG

SEQ ID NO: 14 - protein, 9 aa, synthetic construct
SYGNYPFDY

SEQ ID NO: 15 - protein, 10 aa, synthetic construct
SASSSVSYMY

SEQ ID NO: 16 - protein, 7 aa, synthetic construct
DTSNLAS

SEQ ID NO: 17 - protein, 9 aa, synthetic construct
QQWSSYPLT

SEQ ID NO: 18 - protein, 119 aa, synthetic construct
QVQLVQSGAEVKKPGASVKVSCKASGYSFTSSWIHWVKQAPGQGLEWMGEINPGNVRSNYNENFRNKVTMTVDTSISTAYMELSRLRSDDTAVYYCTVINYGEPYFASWGQGTLVTVSS

SEQ ID NO: 19 - protein, 108 aa, synthetic construct
EIVLTQSPGTLSLSPGERATLSCRASQSVIGSYLAWYQQKPGQAPRLLIYSASKLASGIPDRFSGSGSGTDFTLTISRLEPEDFAVYYCQQDTRYPITFGQGTKVEIK

SEQ ID NO: 20 - protein, 119 aa, synthetic construct
QVQLVQSGAEVKKPGASVKVSCKASGYSFTSSWIHWVRQAPGQGLEWMGEINPGSGRSNYNENFQGRVTMTVDTSISTAYMELSRLRSDDTAVYYCTVVFYGEPYFPFWGQGTLVTVSS

SEQ ID NO: 21 - protein, 108 aa, synthetic construct
EIVLTQSPGTLSLSPGERATLSCRASQSVIYSYLAWYQQKPGQAPRLLIYSASKRASGIPDRFSGSGSGTDFTLTISRLEPEDFAVYYCQQHAGIPVTFGQGTKVEIK

SEQ ID NO: 22 - protein, 118 aa, synthetic construct
EVQLVESGGGLVQPGGSLRLSCAASGFTFSSYAMSWVRQAPGKGLVWVAEISRGGSHTYYPDTVTGRFTISRDNAKNTLYLQMNSLRAEDTAVYYCARSYGNYPFDYWGQGTTVTVSS

SEQ ID NO: 23 - protein, 106 aa, synthetic construct
EIVLTQSPATLSLSPGERATLSCSASSSVSYMYWYQQKPGQAPRLLIYDTSNLASGIPARFSGSGSGTDFTLTISSLEPEDFAVYYCQQWSSYPLTFGQGTKLEIK

SEQ ID NO: 24 - protein, 316 aa, Homo sapiens
DGCKDIFMKNEILSASQPFAFNCTFPPITSGEVSVTWYKNSSKIPVSKIIQSRIHQDETWILFLPMEWGDSGVYQCVIKGRDSCHRIHVNLTVFEKHWCDTSIGGLPNLSDEYKQILHLGKDDSLTCHLHFPKSCVLGPIKWYKDCNEIKGERFTVLETRLLVSNVSAEDRGNYACQAILTHSGKQYEVLNGITVSITERAGYGGSVPKIIYPKNHSIEVQLGTTLIVDCNVTDTKDNTNLRCWRVNNTLVDDYYDESKRIREGVETHVSFREHNLYTVNITFLEVKMEDYGLPFMCHAGVSTAYIILQLPAPDFR

SEQ ID NO: 25 - protein, 316 aa, Macaca fascicularis
DGCNDIFMKNEMLSASQPFAFNCTFPPITSGEVSVTWYKNSSKIPVSKIIQSRIHQDETWILFLPMEWGDSGVYQCVIKGRDSCHRIHVNLTVFEKQWCDTSVKGLPNLSDEYKQILHLGKDDSLTCHLHFPKSCILGPIKWYKDCNEITGERFTVLETRLLVSNVSAEDRGNYACQVILTHSGKQYEVLNGITVSITERAGYGGSVPKIIYPKNNSIEVQLGTTLIVDCNITDTKDNTNLRCWRVNNTLVDDYYNESKRIREGVETHASFREYNLYTVNITFLEVKMEDYGLPFMCHAGVSAAYIMLQLPAPDFR

SEQ ID NO: 26 - protein, 339 aa, Homo sapiens
SERCDDWGLDTMRQIQVFEDEPARIKCPLFEHFLKFNYSTAHSAGLTLIWYWTRQDRDLEEPINFRLPENRISKEKDVLWFRPTLLNDTGNYTCMLRNTTYCSKVAFPLEVVQKDSCFNSPMKLPVHKLYIEYGIQRITCPNVDGYFPSSVKPTITWYMGCYKIQNFNNVIPEGMNLSFLIALISNNGNYTCVVTYPENGRTFHLTRTLTVKVVGSPKNAVPPVIHSPNDHVVYEKEPGEELLIPCTVYFSFLMDSRNEVWWTIDGKKPDDITIDVTINESISHSRTEDETRTQILSIKKVTSEDLKRSYVCHARSAKGEVAKAAKVKQKVPAPRYTVE

SEQ ID NO: 27 - protein, 339 aa, Macaca fascicularis
SERCDDWGLDTMRQIQVFEDEPARIKCPLFEHFLKFNYSTAHSAGLTLIWYWTRQDRDLEEPINFRLPENRISKEKDVLWFRPTLLNDTGNYTCMLRNTTYCSKVAFPLEVVQKDSCFNSPMKLPVHKLYIEYGIQRITCPNVDGYFPSSVKPTITWYMGCYKIQNFNNVIPEGMNLSFLIAFISNNGNYTCVVTYPENGRTFHLTRTLTVKVVGSPKNAVPPVIHSPNDHVVYEKEPGEELLIPCTVYFSFLMDSRNEVWWTIDGKKPDDIPIDVTINESISHSRTEDETRTQILSIKKVTSEDLKRSYVCHARSAKGEVAKAATVKQKVPAPRYTVE

SEQ ID NO: 28 - protein, 159 aa, Homo sapiens
SAPFSFLSNVKYNFMRIIKYEFILNDALNQSIIRANDQYLTAAALHNLDEAVKFDMGAYKSSKDDAKITVILRISKTQLYVTAQDEDQPVLLKEMPEIPKTITGSETNLLFFWETHGTKNYFTSVAHPNLFIATKQDYWVCLAGGPPSITDFQILENQA

SEQ ID NO: 29 - protein, 153 aa, Homo sapiens
APVRSLNCTLRDSQQKSLVMSGPYELKALHLQGQDMEQQVVFSMSFVQGEESNDKIPVALGLKEKNLYLSCVLKDDKPTLQLESVDPKNYPKKKMEKRFVFNKIEINNKLEFESAQFPNWYISTSQAENMPVFLGGTKGGQDITDFTMQFVSS

SEQ ID NO: 30 - protein, 159 aa, Homo sapiens
SITGISPITEYLASLSTYNDQSITFALEDESYEIYVEDLKKDEKKDKVLLSYYESQHPSNESGDGVDGKMLMVTLSPTKDFWLHANNKEHSVELHKCEKPLPDQAFFVLHNMHSNCVSFECKTDPGVFIGVKDNHLALIKVDSSENLCTENILFKLSET

SEQ ID NO: 31 - protein, 153 aa, Homo sapiens
KIDTPQQGSIQDINHRVWVLQDQTLIAVPRKDRMSPVTIALISCRHVETLEKDRGNPIYLGLNGLNLCLMCAKVGDQPTLQLKEKDIMDLYNQPEPVKSFLFYHSQSGRNSTFESVAFPGWFIAVSSEGGCPLILTQELGKANTTDFGLTMLF

SEQ ID NO: 32 - protein, 153 aa, Homo sapiens
REAAPKSYAIRDSRQMVWVLSGNSLIAAPLSRSIKPVTLHLIACRDTEFSDKEKGNMVYLGIKGKDLCLFCAEIQGKPTLQLKEKNIMDLYVEKKAQKPFLFFHNKEGSTSVFQSVSYPGWFIATSTTSGQPIFLTKERGITNNTNFYLDSVE

SEQ ID NO: 33 - protein, 152 aa, Homo sapiens
SMCKPITGTINDLNQQVWTLQGQNLVAVPRSDSVTPVTVAVITCKYPEALEQGRGDPIYLGIQNPEMCLYCEKVGEQPTLQLKEQKIMDLYGQPEPVKPFLFYRAKTGRTSTLESVAFPDWFIASSKRDQPIILTSELGKSYNTAFELNIND

SEQ ID NO: 34 - protein, 6 aa, synthetic construct
HHHHHH

SEQ ID NO: 35 - protein, 232 aa, Mus musculus
PRGPTIKPCPPCKCPAPNLLGGPSVFIFPPKIKDVLMISLSPIVTCVVVDVSEDDPDVQISWFVNNVEVHTAQTQTHREDYNSTLRVVSALPIQHQDWMSGKEFKCKVNNKDLPAPIERTISKPKGSVRAPQVYVLPPPEEEMTKKQVTLTCMVTDFMPEDIYVEWTNNGKTELNYKNTEPVLDSDGSYFMYSKLRVEKKNWVERNSYSCSVVHEGLHNHHTTKSFSRTPGK

SEQ ID NO: 36 - protein, 330 aa, Homo sapiens
ASTKGPSVFPLAPSSKSTSGGTAALGCLVKDYFPEPVTVSWNSGALTSGVHTFPAVLQSSGLYSLSSVVTVPSSSLGTQTYICNVNHKPSNTKVDKRVEPKSCDKTHTCPPCPAPELLGGPSVFLFPPKPKDTLMISRTPEVTCVVVDVSHEDPEVKFNWYVDGVEVHNAKTKPREEQYNSTYRVVSVLTVLHQDWLNGKEYKCKVSNKALPAPIEKTISKAKGQPREPQVYTLPPSREEMTKNQVSLTCLVKGFYPSDIAVEWESNGQPENNYKTTPPVLDSDGSFFLYSKLTVDKSRWQQGNVFSCSVMHEALHNHYTQKSLSLSPGK

SEQ ID NO: 37 - protein, 330 aa, synthetic construct
ASTKGPSVFPLAPSSKSTSGGTAALGCLVKDYFPEPVTVSWNSGALTSGVHTFPAVLQSSGLYSLSSVVTVPSSSLGTQTYICNVNHKPSNTKVDKRVEPKSCDKTHTCPPCPAPEFEGGPSVFLFPPKPKDTLMISRTPEVTCVVVDVSHEDPEVKFNWYVDGVEVHNAKTKPREEQYNSTYRVVSVLTVLHQDWLNGKEYKCKVSNKALPASIEKTISKAKGQPREPQVYTLPPSREEMTKNQVSLTCLVKGFYPSDIAVEWESNGQPENNYKTTPPVLDSDGSFFLYSKLTVDKSRWQQGNVFSCSVMHEALHNHYTQKSLSLSPGK

SEQ ID NO: 38 - protein, 330 aa, synthetic construct
ASTKGPSVFPLAPSSKSTSEGTAALGCLVKDYFPEPVTVSWNSGALTSGVHTFPAVLQSSGLYSLSSVVTVPSSSLGTQTYICNVDHKPSNTKVDKTVEPKSCDKTHTCPPCPAPEFEGGPSVFLFPPKPKDTLMISRTPEVTCVVVDVSQEDPEVQFNWYVDGVEVHNAKTKPREEQYNSTYRVVSVLTVLHQDWLNGKEYKCKVSNKALPASIEKTISKAKGQPREPQVCTLPPSQEEMTKNQVSLSCAVKGFYPSDIAVEWESNGQPENNYKTTPPVLDSDGSFFLVSKLTVDKSRWQEGNVFSCSVMHEALHNHYTQKSLSLSPGK

SEQ ID NO: 39 - protein, 330 aa, synthetic construct
ASTKGPSVFPLAPSSKSTSGGTAALGCLVKDYFPEPVTVSWNSGALTSGVHTFPAVLQSSGLYSLSSVVTVPSSSLGTQTYICNVNHKPSNTKVDKRVEPKSCDKTHTCPPCPAPEFEGGPSVFLFPPKPKDTLMISRTPEVTCVVVDVSHEDPEVKFNWYVDGVEVHNAKTKPREEQYNSTYRVVSVLTVLHQDWLNGKEYKCKVSNKALPASIEKTISKAKGQPREPQVYTLPPCREEMTKNQVSLWCLVKGFYPSDIAVEWESNGQPENNYKTTPPVLDSDGSFFLYSKLTVDKSRWQQGNVFSCSVMHEALHNHYTQKSLSLSPGK

SEQ ID NO: 40 - protein, 107 aa, Homo sapiens [sequence omitted]

SEQ ID NO: 41 - protein, 106 aa, Homo sapiens
GQPKAAPSVTLFPPSSEELQANKATLVCLISDFYPGAVTVAWKADSSPVKAGVETTTPSKQSNNKYAASSYLSLTPEQWKSHRSYSCQVTHEGSTVEKTVAPTECS

SEQ ID NO: 42 - protein, 119 aa, synthetic construct [sequence omitted]

SEQ ID NO: 43 - protein, 108 aa, synthetic construct [sequence omitted]

SEQ ID NO: 44 - protein, 449 aa, synthetic construct
QVQLVQSGAEVKKPGASVKVSCKASGYSFTSSWIHWVRQAPGQGLEWMGEINPGSGRSNYNENFQGRVTMTVDTSISTAYMELSRLRSDDTAVYYCTVVFYGEPYFPFWGQGTLVTVSSASTKGPSVFPLAPSSKSTSEGTAALGCLVKDYFPEPVTVSWNSGALTSGVHTFPAVLQSSGLYSLSSVVTVPSSSLGTQTYICNVDHKPSNTKVDKTVEPKSCDKTHTCPPCPAPEFEGGPSVFLFPPKPKDTLMISRTPEVTCVVVDVSQEDPEVQFNWYVDGVEVHNAKTKPREEQYNSTYRVVSVLTVLHQDWLNGKEYKCKVSNKALPASIEKTISKAKGQPREPQVCTLPPSQEEMTKNQVSLSCAVKGFYPSDIAVEWESNGQPENNYKTTPPVLDSDGSFFLVSKLTVDKSRWQEGNVFSCSVMHEALHNHYTQKSLSLSPGK

SEQ ID NO: 45 - protein, 448 aa, synthetic construct
EVQLVESGGGLVQPGGSLRLSCAASGFTFSSYAMSWVRQAPGKGLVWVAEISRGGSHTYYPDTVTGRFTISRDNAKNTLYLQMNSLRAEDTAVYYCARSYGNYPFDYWGQGTTVTVSSASTKGPSVFPLAPSSKSTSGGTAALGCLVKDYFPEPVTVSWNSGALTSGVHTFPAVLQSSGLYSLSSVVTVPSSSLGTQTYICNVNHKPSNTKVDKRVEPKSCDKTHTCPPCPAPEFEGGPSVFLFPPKPKDTLMISRTPEVTCVVVDVSHEDPEVKFNWYVDGVEVHNAKTKPREEQYNSTYRVVSVLTVLHQDWLNGKEYKCKVSNKALPASIEKTISKAKGQPREPQVYTLPPCREEMTKNQVSLWCLVKGFYPSDIAVEWESNGQPENNYKTTPPVLDSDGSFFLYSKLTVDKSRWQQGNVFSCSVMHEALHNHYTQKSLSLSPGK

SEQ ID NO: 46 - protein, 215 aa, synthetic construct
EIVLTQSPGTLSLSPGERATLSCRASQSVIGSYLAWYQQKPGQAPRLLIYSASKLASGIPDRFSGSGSGTDFTLTISRLEPEDFAVYYCQQDTRYPITFGQGTKVEIKRTVAAPSVFIFPPSDEQLKSGTASVVCLLNNFYPREAKVQWKVDNALQSGNSQESVTEQDSKDSTYSLSSTLTLSKADYEKHKVYACEVTHQGLSSPVTKSFNRGEC

SEQ ID NO: 47 - protein, 215 aa, synthetic construct
EIVLTQSPGTLSLSPGERATLSCRASQSVIYSYLAWYQQKPGQAPRLLIYSASKRASGIPDRFSGSGSGTDFTLTISRLEPEDFAVYYCQQHAGIPVTFGQGTKVEIKRTVAAPSVFIFPPSDEQLKSGTASVVCLLNNFYPREAKVQWKVDNALQSGNSQESVTEQDSKDSTYSLSSTLTLSKADYEKHKVYACEVTHQGLSSPVTKSFNRGEC

SEQ ID NO: 48 - protein, 452 aa, synthetic construct
EVQLVESGGGLVQPGGSLRLSCAASGFTFSSYAMSWVRQAPGKGLVWVAEISRGGSHTYYPDTVTGRFTISRDNAKNTLYLQMNSLRAEDTAVYYCARSYGNYPFDYWGQGTTVTVSSASVAAPSVFIFPPSDEQLKSGTASVVCLLNNFYPREAKVQWKVDNALQSGNSQESVTEQDSKDSTYSLSSTLTLSKADYEKHKVYACEVTHQGLSSPVTKSFNRGECDKTHTCPPCPAPEFEGGPSVFLFPPKPKDTLMISRTPEVTCVVVDVSHEDPEVKFNWYVDGVEVHNAKTKPREEQYNSTYRVVSVLTVLHQDWLNGKEYKCKVSNKALPASIEKTISKAKGQPREPQVYTLPPCREEMTKNQVSLWCLVKGFYPSDIAVEWESNGQPENNYKTTPPVLDSDGSFFLYSKLTVDKSRWQQGNVFSCSVMHEALHNHYTQKSLSLSPGK

SEQ ID NO: 49 - protein, 211 aa, synthetic construct
EIVLTQSPATLSLSPGERATLSCSASSSVSYMYWYQQKPGQAPRLLIYDTSNLASGIPARFSGSGSGTDFTLTISSLEPEDFAVYYCQQWSSYPLTFGQGTKLEIKSSASTKGPSVFPLAPSSKSTSGGTAALGCLVKDYFPEPVTVSWNSGALTSGVHTFPAVLQSSGLYSLSSVVTVPSSSLGTQTYICNVNHKPSNTKVDKRVEPKSC

SEQ ID NO: 50 - protein, 449 aa, synthetic construct
QVQLVQSGAEVKKPGASVKVSCKASGYSFTSSWIHWVKQAPGQGLEWMGEINPGNVRSNYNENFRNKVTMTVDTSISTAYMELSRLRSDDTAVYYCTVINYGEPYFASWGQGTLVTVSSASTKGPSVFPLAPSSKSTSEGTAALGCLVKDYFPEPVTVSWNSGALTSGVHTFPAVLQSSGLYSLSSVVTVPSSSLGTQTYICNVDHKPSNTKVDKTVEPKSCDKTHTCPPCPAPEFEGGPSVFLFPPKPKDTLMISRTPEVTCVVVDVSQEDPEVQFNWYVDGVEVHNAKTKPREEQYNSTYRVVSVLTVLHQDWLNGKEYKCKVSNKALPASIEKTISKAKGQPREPQVCTLPPSQEEMTKNQVSLSCAVKGFYPSDIAVEWESNGQPENNYKTTPPVLDSDGSFFLVSKLTVDKSRWQEGNVFSCSVMHEALHNHYTQKSLSLSPGK

SEQ ID NO: 51 - protein, 118 aa, synthetic construct
EVKLVESGGGLVKPGGSLKLSCAASGFTFSSYAMSWVRQSPEKRLEWVAEISRGGSHTYYPDTVTGRFTISRDNAKNTLYLEMTSLRSEDTALYYCARSYGNYPFDYWGQGTTLTVSS

SEQ ID NO: 52 - protein, 106 aa, synthetic construct
DIVMTQSPAIMSASPGEKVTMTCSASSSVSYMYWYQQKPGSSPRLLIYDTSNLASGVPVRFSGSGSGTSYSLTISRMEAEDAATYYCQQWSSYPLTFGAGTKLEIK

SEQ ID NO: 53 - protein, 115 aa, synthetic construct
EVQLLESGGGLVQPGGSLRLSCAASGFTFSSYAMSWVRQAPGKGLEWVSAISGSGGSTYYADSVKGRFTISRDNSKNTLYLQMNSLRAEDTAVYYCAKGSGFDYWGQGTLVTVSS

SEQ ID NO: 54 - protein, 108 aa, synthetic construct
EIVLTQSPGTLSLSPGERATLSCRASQSVSSSYLAWYQQKPGQAPRLLIYGASSRATGIPDRFSGSGSGTDFTLTISRLEPEDFAVYYCQQYGSSPLTFGQGTKVEIK

SEQ ID NO: 55 - DNA, 19 bp, synthetic construct
  source 1..19: mol_type = other DNA
tgcatttgaactccttgcc

SEQ ID NO: 56 - DNA, 20 bp, synthetic construct
  source 1..20: mol_type = other DNA
ccatcaatcttccacttgac